European Patent Specification EP 3 656 849 B1, published January 1, 2025. Title: IN VITRO PRODUCTION OF MEDIAL GANGLIONIC EMINENCE PRECURSOR CELLS. Applicant: THE REGENTS OF THE UNIVERSITY OF CALIFORNIA. Application EP. The sequence listing filed with the application follows.

SEQUENCE LISTING (28 sequences)

SEQ ID NO: 1 - DNA, 20 bp, Artificial sequence
  Synthetic Oligonucleotide
gtcctgtcgcccaccatctc

SEQ ID NO: 2 - DNA, 19 bp, Artificial sequence
  Synthetic Oligonucleotide
ccctcccaacgccactgac

SEQ ID NO: 3 - DNA, 21 bp, Artificial sequence
  Synthetic Oligonucleotide
tcagagatgtcccgactcctg

SEQ ID NO: 4 - DNA, 22 bp, Artificial sequence
  Synthetic Oligonucleotide
gccgcttctatccttgtcgtaa

SEQ ID NO: 5 - DNA, 21 bp, Artificial sequence
  Synthetic Oligonucleotide
gcctcaacaacgtcccttact

SEQ ID NO: 6 - DNA, 23 bp, Artificial sequence
  Synthetic Oligonucleotide
tcactatccgaatttcaggctca

SEQ ID NO: 7 - DNA, 21 bp, Artificial sequence
  Synthetic Oligonucleotide
agaagaacggcaagtacgaga

SEQ ID NO: 8 - DNA, 21 bp, Artificial sequence
  Synthetic Oligonucleotide
tgttgagggacagattgtggc

SEQ ID NO: 9 - DNA, 22 bp, Artificial sequence
  Synthetic Oligonucleotide
cgaggactctggacagtagagg

SEQ ID NO: 10 - DNA, 22 bp, Artificial sequence
  Synthetic Oligonucleotide
gatcttgagccccagttttctg

SEQ ID NO: 11 - DNA, 22 bp, Artificial sequence
  Synthetic Oligonucleotide
ggtggtctcctctgacttcaac

SEQ ID NO: 12 - DNA, 22 bp, Artificial sequence
  Synthetic Oligonucleotide
ttcgttgtcataccaggaaatg

SEQ ID NO: 13 - DNA, 23 bp, Artificial sequence
  Synthetic Oligonucleotide
tctgcaagatggactacttcagc

SEQ ID NO: 14 - DNA, 21 bp, Artificial sequence
  Synthetic Oligonucleotide
cttgggttgactgtcctgttc

SEQ ID NO: 15 - DNA, 20 bp, Artificial sequence
  Synthetic Oligonucleotide
agactcgctcgctcatttgt

SEQ ID NO: 16 - DNA, 20 bp, Artificial sequence
  Synthetic Oligonucleotide
ctccatgcccactttcttgt

SEQ ID NO: 17 - DNA, 20 bp, Artificial sequence
  Synthetic Oligonucleotide
cgctgcgacactacatcaac

SEQ ID NO: 18 - DNA, 20 bp, Artificial sequence
  Synthetic Oligonucleotide
cagggtcttcaagccgagtt

SEQ ID NO: 19 - DNA, 19 bp, Artificial sequence
  Synthetic Oligonucleotide
agctcctcaaatcgcatcc

SEQ ID NO: 20 - DNA, 19 bp, Artificial sequence
  Synthetic Oligonucleotide
atagtcgtcgcagctttcg

SEQ ID NO: 21 - DNA, 21 bp, Artificial sequence
  Synthetic Oligonucleotide
gcaaaacccggaggaggagtc

SEQ ID NO: 22 - DNA, 21 bp, Artificial sequence
  Synthetic Oligonucleotide
ccacatcggcctgtgtatatc

SEQ ID NO: 23 - DNA, 22 bp, Artificial sequence
  Synthetic Oligonucleotide
aaagagtgcggatgatgtgaag

SEQ ID NO: 24 - DNA, 19 bp, Artificial sequence
  Synthetic Oligonucleotide
accccaattttgccgtccc

SEQ ID NO: 25 - DNA, 19 bp, Artificial sequence
  Synthetic Oligonucleotide
gctgctgtctgaacccaac

SEQ ID NO: 26 - DNA, 19 bp, Artificial sequence
  Synthetic Oligonucleotide
cgttctcggggtgccatag

SEQ ID NO: 27 - DNA, 18 bp, Artificial sequence
  Synthetic Oligonucleotide
gcaactacgtgggcgact

SEQ ID NO: 28 - DNA, 20 bp, Artificial sequence
  Synthetic Oligonucleotide
cgaggcacgtacttgtgaga